European Patent Application EP 4 356 970 A1, published April 24, 2024. Title: PREPARATION AND APPLICATION OF LOX1-BASED CHIMERIC ANTIGEN RECEPTOR IMMUNE CELL. Applicant: WEST CHINA HOSPITAL, SICHUAN UNIVERSITY. The sequence listing filed with the application follows.

SEQUENCE LISTING (9 sequences)

SEQ ID NO: 1 - protein, 273 aa, Homo sapiens
MTFDDLKIQTVKDQPDEKSNGKKAKGLQFLYSPWWCLAAATLGVLCLGLVVTIMVLGMQLSQVSDLLTQEQANLTHQKKKLEGQISARQQAEEASQESENELKEMIETLARKLNEKSKEQMELHHQNLNLQETLKRVANCSAPCPQDWIWHGENCYLFSSGSFNWEKSQEKCLSLDAKLLKINSTADLDFIQQAISYSSFPFWMGLSRRNPSYPWLWEDGSPLMPHLFRVRGAVSQTYPSGTCAYIQRGAVYAENCILAAFSICQKKANLRAQ

SEQ ID NO: 2 - protein, 233 aa, Artificial sequence
  mKate2 red fluorescent protein
MSELIKENMHMKLYMEGTVNNHHFKCTSEGEGKPYEGTQTMRIKAVEGGPLPFAFDILATSFMYGSKTFINHTQGIPDFFKQSFPEGFTWERVTTYEDGGVLTATQDTSLQDGCLIYNVKIRGVNFPSNGPVMQKKTLGWEASTETLYPADGGLEGRADMALKLVGGGHLICNLKTTYRSKKPAKNLKMPGVYYVDRRLERIKEADKETYVEQHEVAVARYCDLPSKLGHKLN

SEQ ID NO: 3 - protein, 22 aa, Artificial sequence
  signal peptide
MAAATGPSFWLGNETLKVPLAL

SEQ ID NO: 4 - protein, 45 aa, Artificial sequence
  CD8 hinge
TTTPAPRPPTPAPTIASQPLSLRPEACRPAAGGAVHTRGLDFACD

SEQ ID NO: 5 - protein, 24 aa, Artificial sequence
  CD28 transmembrane region
IYIWAPLAGTCGVLLLSLVITLYC

SEQ ID NO: 6 - protein, 43 aa, Artificial sequence
  costimulatory molecule derived from 4-1BB
KRGRKKLLYIFKQPFMRPVQTTQEEDGCSCRFPEEEEGGCELR

SEQ ID NO: 7 - protein, 111 aa, Artificial sequence
  cytoplasmic signaling sequence derived from CD3zeta
VKFSRSADAPAYKQGQNQLYNELNLGRREEYDVLDKRRGRDPEMGGKPRRKNPQEGLYNELQKDKMAEAYSEIGMKGERRRGKGHDGLYQGLSTATKDTYDALHMQALPPR

SEQ ID NO: 8 - protein, 439 aa, Artificial sequence
  full length of CAR
MQLSQVSDLLTQEQANLTHQKKKLEGQISARQQAEEASQESENELKEMIETLARKLNEKSKEQMELHHQNLNLQETLKRVANCSAPCPQDWIWHGENCYLFSSGSFNWEKSQEKCLSLDAKLLKINSTADLDFIQQAISYSSFPFWMGLSRRNPSYPWLWEDGSPLMPHLFRVRGAVSQTYPSGTCAYIQRGAVYAENCILAAFSICQKKANLRAQTTTPAPRPPTPAPTIASQPLSLRPEACRPAAGGAVHTRGLDFACDIYIWAPLAGTCGVLLLSLVITLYCKRGRKKLLYIFKQPFMRPVQTTQEEDGCSCRFPEEEEGGCELRVKFSRSADAPAYKQGQNQLYNELNLGRREEYDVLDKRRGRDPEMGGKPRRKNPQEGLYNELQKDKMAEAYSEIGMKGERRRGKGHDGLYQGLSTATKDTYDALHMQALPPR

SEQ ID NO: 9 - DNA, 1317 bp, Artificial sequence
  full length of CAR
atgcaattatcccaggtgtctgacctcctaacacaagagcaagcaaacctaactcaccagaaaaagaaactggagggacagatctcagcccggcaacaagcagaagaagcttcacaggagtcagaaaacgaactcaaggaaatgatagaaacccttgctcggaagctgaatgagaaatccaaagagcaaatggaacttcaccaccagaatctgaatctccaagaaacactgaagagagtagcaaattgttcagctccttgtccgcaagactggatctggcatggagaaaactgttacctattttcctcgggctcatttaactgggaaaagagccaagagaagtgcttgtctttggatgccaagttgctgaaaattaatagcacagctgatctggacttcatccagcaagcaatttcctattccagttttccattctggatggggctgtctcggaggaaccccagctacccatggctctgggaggacggttctcctttgatgccccacttatttagagtccgaggcgctgtctcccagacatacccttcaggtacctgtgcatatatacaacgaggagctgtttatgcggaaaactgcattttagctgccttcagtatatgtcagaagaaggcaaacctaagagcacagaccacgacgccagcgccgcgaccaccaacaccggcgcccaccatcgctagccagcccctgtccctgcgcccagaggcgtgccggccagcggcggggggcgcagtgcacacgagggggctggacttcgcctgtgatatctacatctgggcgcccttggccgggacttgtggggtccttctcctgtcactggttatcaccctttactgcaaacggggcagaaagaaactcctgtatatattcaaacaaccatttatgagaccagtacaaactactcaagaggaagatggctgtagctgccgatttccagaagaagaagaaggaggatgtgaactgagagtgaagttcagcaggagcgcagacgcccccgcgtacaagcagggccagaaccagctctataacgagctcaatctaggacgaagagaggagtacgatgttttggacaagagacgtggccgggaccctgagatggggggaaagccgagaaggaagaaccctcaggaaggcctgtacaatgaactgcagaaagataagatggcggaggcctacagtgagattgggatgaaaggcgagcgccggaggggcaaggggcacgatggcctttaccagggtctcagtacagccaccaaggacacctacgacgcccttcacatgcaggccctgccccctcgc